European Patent Specification EP 3 986 890 B1, published November 15, 2023. Title: Benzisoxazole Sulfonamide Derivatives. Applicant: Pfizer Inc. CTXT PTY LTD. The sequence listing filed with the application follows.

SEQUENCE LISTING (7 sequences)

SEQ ID NO: 1 - protein, 20 aa, Homo sapiens
ARTKQTARKSTGGKAPRKQL

SEQ ID NO: 2 - protein, 20 aa, Homo sapiens
SGRGKGGKGLGKGGAKRHRK

SEQ ID NO: 3 - protein, 21 aa, Homo sapiens
ARTKQTARKSTGGKAPRKQLA

SEQ ID NO: 4 - protein, 21 aa, Homo sapiens
SGRGKGGKGLGKGGAKRHRKV

SEQ ID NO: 5 - protein, 480 aa, Artificial Sequence
  modified KAT5 protein
MGHHHHHHGTENLYFQGSAEVGEIIEGCRLPVLRRNQDNEDEWPLAEILSVKDISGRKLFYVHYIDFNKRLDEWVTHERLDLKKIQFPKKEAKTPTKNGLPGSRPGSPEREVKRKVEVVSPATPVPSETAPASVFPQNGAARRAVAAQPGRKRKSNCLGTDEDSQDSSDGIPSAPRMTGSLVSDRSHDDIVTRMKNIECIELGRHRLKPWYFSPYPQELTTLPVLYLCEFCLKYGRSLKCLQRHLTKCDLRHPPGNEIYRKGTISFFEIDGRKNKSYSQNLCLLAKCFLDHKTLYYDTDPFLFYVMTEYDCKGFHIVGYFSKEKESTEDYNVACILTLPPYQRRGYGKLLIEFSYELSKVEGKTGTPEKPLSDLGLLSYRSYWSQTILEILMGLKSESGERPQITINEISEITSIKKEDVISTLQYLNLINYYKGQYILTLSEDIVDGHERAMLKRLLRIDSKCLHFTPKDWSKRGKWAS

SEQ ID NO: 6 - protein, 791 aa, Artificial Sequence
  modified KAT6A protein
MNKEILAVVEAVSNEKALPREKIFEALESALATATKKKYEQEIDVRVQIDRKSGDFDTFRRWLVVDEVTQPTKEITLEAARYEDESLNLGDYVEDQIESVTFDRITTQTAKQVIVQKVREAERAMVVDQFREHEGEIITGVVKKVNRDNISLDLGNNAEAVILREDMLPRENFRPGDRVRGVLYSVRPEARGAQLFVTRSKPEMLIELFRIEVPEIGEEVIEIKAAARDPGSRAKIAVKTNDKRIDPVGACVGMRGARVQAVSTELGGERIDIVLWDDNPAQFVINAMAPADVASIVVDEDKHTMDIAVEAGNLAQAIGRNGQNVRLASQLSGWELNVMTVDDLQAKHQAEAHAAIDTFTKYLDIDEDFATVLVEEGFSTLEELAYVPMKELLEIEGLDEPTVEALRERAKNALATIAQAQEESLGDNKPADDLLNLEGVDRDLAFKLAARGVCTLEDLAEQGIDDLADIEGLTDEKAGALIMAARNICWFGDEATSGSGHHHHHHSAGENLYFQGAMGRCPSVIEFGKYEIHTWYSSPYPQEYSRLPKLYLCEFCLKYMKSRTILQQHMKKCGWFHPPVNEIYRKNNISVFEVDGNVSTIYCQNLCLLAKLFLDHKTLYYDVEPFLFYVLTQNDVKGCHLVGYFSKEKHCQQKYNVSCIMILPQYQRKGYGRFLIDFSYLLSKREGQAGSPEKPLSDLGRLSYMAYWKSVILECLYHQNDKQISIKKLSKLTGICPQDITSTLHHLRMLDFRSDQFVIIRREKLIQDHMAKLQLNLRPVDVDPECLRWTP

SEQ ID NO: 7 - protein, 307 aa, Artificial Sequence
  modified KAT7 protein
MGHHHHHHGTENLYFQGSRLQGQITEGSNMIKTIAFGRYELDTWYHSPYPEEYARLGRLYMCEFCLKYMKSQTILRRHMAKCVWKHPPGDEIYRKGSISVFEVDGKKNKIYCQNLCLLAKLFLDHKTLYYDVEPFLFYVMTEADNTGCHLIGYFSKEKNSFLNYNVSCILTMPQYMRQGYGKMLIDFSYLLSKVEEKVGSPERPLSDLGLISYRSYWKEVLLRYLHNFQGKEISIKEISQETAVNPVDIVSTLQALQMLKYWKGKHLVLKRQDLIDEWIAKEAKRSNSNKTMDPSCLKWTPPKGTAS